European Patent Specification EP 3 610 887 B1, published November 15, 2023. Title: Compositions and Methods of Enhancing Immune Responses to Eimeria or Limiting Eimeria Infection. Applicant: The Board of Trustees of the University of Arkansas The Texas A&M University System. Application EP. The sequence listing filed with the application follows.

SEQUENCE LISTING (40 sequences)

SEQ ID NO: 1 - protein, 16 aa, Artificial sequence
  Synthetic: composite minimal epitope
  misc_feature (2)..(2): Xaa is Arg or Met
  misc_feature (3)..(4): Xaa is Val or Ile
  misc_feature (5)..(5): Xaa is Ser or Arg
  misc_feature (6)..(6): Xaa is Phe or Tyr
  misc_feature (13)..(13): Xaa is His or Tyr
PXXXXXGYGACEXNLG

SEQ ID NO: 2 - protein, 43 aa, Eimeria maxima
  misc_feature (1)..(43): Eimeria maxima MPP
PSHDAPESERTPRVISFGYGACEHNLGVSLFRREETKKDPRGR

SEQ ID NO: 3 - protein, 28 aa, Neospora canium
PRIVSFGYGACEHNLGMSLYDRQGLQRQ

SEQ ID NO: 4 - protein, 21 aa, Eimeria tenella
ESQRAPMVIRYGYGACEYNLG

SEQ ID NO: 5 - protein, 10 aa, Eimeria maxima
  misc_feature (1)..(10): Eimeria maxima TRAP-1
GGGFPTAAVA

SEQ ID NO: 6 - protein, 40 aa, Eimeria maxima
  misc_feature (1)..(40): Eimeria maxima TRAP-02
AAPETPAVQPKPEEGHERPEPEEEEEKKEEGGGFPTAAVA

SEQ ID NO: 7 - protein, 40 aa, Eimeria maxima
  misc_feature (1)..(40): Eimeria maxima TRAP-03
GGGFPTAAVAGGVGGVLLIAAVGGGVAAFTSGGGGAGAQE

SEQ ID NO: 8 - protein, 70 aa, Eimeria maxima
  misc_feature (1)..(70): Eimeria maxima TRAP
AAPETPAVQPKPEEGHERPEPEEEEEKKEEGGGFPTAAVAGGVGGVLLIAAVGGGVAAFTSGGGGAGAQE

SEQ ID NO: 9 - protein, 8 aa, Avian Influenza
  misc_feature (1)..(8): Avian Influenza virus m2e
EVETPIRN

SEQ ID NO: 10 - protein, 8 aa, Avian Influenza
  misc_feature (1)..(8): Avian Influenza virus m2e
EVETPTRN

SEQ ID NO: 11 - protein, 12 aa, Avian Influenza
  misc_feature (1)..(12): Avian Influenza virus HA5 UA
LLSRINHFEKIQ

SEQ ID NO: 12 - protein, 19 aa, Avian Influenza
  misc_feature (1)..(19): Avian Influenza virus HA5 LB
ANPANDLCYPGDFNDYEEL

SEQ ID NO: 13 - protein, 16 aa, Avian Influenza
  misc_feature (1)..(16): Avian Influenza virus NP 54-69
GRLIQNSITIERMVLS

SEQ ID NO: 14 - protein, 14 aa, Avian Influenza
  misc_feature (1)..(14): Avian Influenza virus NP 147-160
TYQRTRALVRTGMD

SEQ ID NO: 15 - protein, 190 aa, Gallus gallus
  misc_feature (1)..(190): Chicken HMGB1 amino acid
MGKGDPKKPRGKMSSYAFFVQTCREEHKKKHPDASVNFSEFSKKCSERWKTMSSKEKGKFEDMAKADKLRYEKEMKNYVPPKGETKKKFKDPNAPKRPPSAFFLFCSEFRPKIKGEHPGLSIGDVAKKLGEMWNNTAADDKQPYEKKAAKLKEKYEKDIAAYRAKGKVDAGKKVVAKAEKSKKKKEEEED

SEQ ID NO: 16 - protein, 85 aa, Artificial sequence
  Synthetic: HMGB1 box a1
MGKGDPKKPRGKMSSYAFFVQTCREEHKKKHPDASVNFSEFSKKCSERWKTMSSKEKGKFEDMAKADKLRYEKEMKNYVPPKGET

SEQ ID NO: 17 - protein, 54 aa, Artificial sequence
  Synthetic: HMGB1 box a2
PDASVNFSEFSKKCSERWKTMSSKEKGKFEDMAKADKLRYEKEMKNYVPPKGET

SEQ ID NO: 18 - protein, 73 aa, Artificial sequence
  Synthetic: HMGB1 box b1
KDPNAPKRPPSAFFLFCSEFRPKIKGEHPGLSIGDVAKKLGEMWNNTAADDKQPYEKKAAKLKEKYEKDIAAY

SEQ ID NO: 19 - protein, 69 aa, Artificial sequence
  Synthetic: HMGB1 box b2
NAPKRPPSAFFLFCSEFRPKIKGEHPGLSIGDVAKKLGEMWNNTAADDKQPYEKKAAKLKEKYEKDIAA

SEQ ID NO: 20 - protein, 21 aa, Artificial sequence
  Synthetic: HMGB1 RAGE Binding domain
KDPNAPKRPPSAFFLFCSEFR

SEQ ID NO: 21 - protein, 33 aa, Artificial sequence
  Synthetic: HMGB1 proinflammatory cytokine activity
LKEKYEKDIAAYRAKGKVDAGKKVVAKAEKSKK

SEQ ID NO: 22 - protein, 215 aa, Homo sapiens
  misc_feature (1)..(215): HMGB1
MGKGDPKKPRGKMSSYAFFVQTCREEHKKKHPDASVNFSEFSKKCSERWKTMSAKEKGKFEDMAKADKARYEREMKTYIPPKGETKKKFKDPNAPKRPPSAFFLFCSEYRPKIKGEHPGLSIGDVAKKLGEMWNNTAADDKQPYEKKAAKLKEKYEKDIAAYRAKGKPDAAKKGVVKAEKSKKKKEEEEDEEDEEDEEEEEDEEDEDEEEDDDDE

SEQ ID NO: 23 - protein, 205 aa, Danio rerio
  misc_feature (1)..(205): Zebra fish HMGB1
MGKDPTKPRGKMSSYAYFVQTCREEHKKKHPEATVNFSEFSKKCSERWKTMSAKEKGKFEDMAKLDKARYEREMKNYIPPKGEKKKRFKDPNAPKRPPSAFFIFCSEFRPKVKEETPGLSIGDVAKRLGEMWNKISSEEKQPYEKKAAKLKEKYEKDIAAYRSKGKVGGGAAKAPSKPDKANDEDEDDDEEEDEDDDDEEEEDDE

SEQ ID NO: 24 - protein, 272 aa, Gallus gallus
  misc_feature (1)..(272): CD154 chicken
MNEAYSPAAPRPMGSTSPSTMKMFMCFLSVFMVVQTIGTVLFCLYLHMKMDKMEEVLSLNEDYIFLRKVQKCQTGEDQKSTLLDCEKVLKGFQDLQCKDRTASEELPKFEMHRGHEHPHLKSRNETSVAEEKRQPIATHLAGVKSNTTVRVLKWMTTSYAPTSSLISYHEGKLKVEKAGLYYIYSQVSFCTKAAASAPFTLYIYLYLPMEEDRLLMKGLDTHSTSTALCELQSIREGGVFELRQGDMVFVNVTDSTAVNVNPGNTYFGMFKL

SEQ ID NO: 25 - protein, 261 aa, Homo sapiens
  misc_feature (1)..(261): Human CD154
MIETYNQTSPRSAATGLPISMKIFMYLLTVFLITQMIGSALFAVYLHRRLDKIEDERNLHEDFVFMKTIQRCNTGERSLSLLNCEEIKSQFEGFVKDIMLNKEETKKENSFEMQKGDQNPQIAAHVISEASSKTTSVLQWAEKGYYTMSNNLVTLENGKQLTVKRQGLYYIYAQVTFCSNREASSQAPFIASLCLKSPGRFERILLRAANTHSSAKPCGQQSIHLGGVFELQPGASVFVNVTDPSQVSHGTGFTSFGLLKL

SEQ ID NO: 26 - protein, 11 aa, Homo sapiens
  misc_feature (1)..(11): Human CD154 peptide
WAEKGYYTMSC

SEQ ID NO: 27 - protein, 11 aa, Gallus gallus
  misc_feature (1)..(11): Chicken CD154 peptide
WMTTSYAPTSS

SEQ ID NO: 28 - protein, 10 aa, Anas sp.
  misc_feature (1)..(10): Duck CD154 peptide
WNKTSYAPMN

SEQ ID NO: 29 - protein, 10 aa, Mus sp.
  misc_feature (1)..(10): Mouse CD154 peptide
WAKKGYYTMK

SEQ ID NO: 30 - protein, 10 aa, Bos taurus
  misc_feature (1)..(10): Cow CD154 peptide
WAPKGYYTLS

SEQ ID NO: 31 - DNA, 918 bp, Artificial sequence
  Synthetic: TRAP MPP HMGB1 nucleotide sequence
ggatccatgggcggtagcagcagaagcagcgcagcacctgaaacgagagcagtccagccgaaacctgaagaaggccatgaaagacctgaacctgaagaagaagaagagaaaaaagaagaaggcggcggctttcctacagcagcagtcgcgggcggatcaagcagatcttccccttctcatgatgcgcctgaaagcgaacggacgcctcgggttatctcctttggttacggtgcgtgcgaacataatctgggcgtctctctttttagacgcgaagaaacgaaaaaagatccgcgtggacggggcggatcaagcagatcttccatgggtaaaggcgacccgaaaaaacctcggggcaaaatgtcaagctacgcatttttcgtccaaacatgcagagaagaacataagaaaaaacatcctgatgctagcgtaaacttttcagaatttagcaaaaaatgttctgaacgttggaaaacgatgtcttccaaagaaaagggtaaatttgaagatatggctaaagccgacaaattgcggtacgaaaaagaaatgaaaaactacgtaccgcctaaaggagaaacaaagaaaaaatttaaagatccgaacgcccctaaaagaccgccttctgcatttttcctgttttgctccgaatttcgcccgaaaattaaaggagaacatcctggtctgagcatcggcgacgttgcgaaaaaacttggagaaatgtggaataacacggcagcggatgacaaacagccgtatgagaaaaaagctgccaaattgaaagaaaaatacgaaaaagatatcgcagcgtaccgcgcaaaaggaaaagtggacgcgggtaaaaaagttgtggctaaagcggaaaaatcaaagaagaaaaaggaagaagaagaagacggcggctcatctcggtcctccgacgtc

SEQ ID NO: 32 - protein, 306 aa, Artificial sequence
  Synthetic: TRAP MPP HMGB1 peptide
GSMGGSSRSSAAPETRAVQPKPEEGHERPEPEEEEEKKEEGGGFPTAAVAGGSSRSSPSHDAPESERTPRVISFGYGACEHNLGVSLFRREETKKDPRGRGGSSRSSMGKGDPKKPRGKMSSYAFFVQTCREEHKKKHPDASVNFSEFSKKCSERWKTMSSKEKGKFEDMAKADKLRYEKEMKNYVPPKGETKKKFKDPNAPKRPPSAFFLFCSEFRPKIKGEHPGLSIGDVAKKLGEMWNNTAADDKQPYEKKAAKLKEKYEKDIAAYRAKGKVDAGKKVVAKAEKSKKKKEEEEDGGSSRSSDV

SEQ ID NO: 33 - DNA, 777 bp, Artificial sequence
  Synthetic: MPP HMGB1 nucleotide
ggatccatgggcggtagcagcagaagcagcccttctcatgatgcgcctgaaagcgaacggacgcctcgggttatctcctttggttacggtgcgtgcgaacataatctgggcgtctctctttttagacgcgaagaaacgaaaaaagatccgcgtggacggggcggatcaagcagatcttccatgggtaaaggcgacccgaaaaaacctcggggcaaaatgtcaagctacgcatttttcgtccaaacatgcagagaagaacataagaaaaaacatcctgatgctagcgtaaacttttcagaatttagcaaaaaatgttctgaacgttggaaaacgatgtcttccaaagaaaagggtaaatttgaagatatggctaaagccgacaaattgcggtacgaaaaagaaatgaaaaactacgtaccgcctaaaggagaaacaaagaaaaaatttaaagatccgaacgcccctaaaagaccgccttctgcatttttcctgttttgctccgaatttcgcccgaaaattaaaggagaacatcctggtctgagcatcggcgacgttgcgaaaaaacttggagaaatgtggaataacacggcagcggatgacaaacagccgtatgagaaaaaagctgccaaattgaaagaaaaatacgaaaaagatatcgcagcgtaccgcgcaaaaggaaaagtggacgcgggtaaaaaagttgtggctaaagcggaaaaatcaaagaagaaaaaggaagaagaagaagacggcggctcatctcggtcctccgacgtc

SEQ ID NO: 34 - protein, 259 aa, Artificial sequence
  Synthetic: MPP HMGB1 peptide
GSMGGSSRSSPSHDAPESERTPRVISFGYGACEHNLGVSLFRREETKKDPRGRGGSSRSSMGKGDPKKPRGKMSSYAFFVQTCREEHKKKHPDASVNFSEFSKKCSERWKTMSSKEKGKFEDMAKADKLRYEKEMKNYVPPKGETKKKFKDPNAPKRPPSAFFLFCSEFRPKIKGEHPGLSIGDVAKKLGEMWNNTAADDKQPYEKKAAKLKEKYEKDIAAYRAKGKVDAGKKVVAKAEKSKKKKEEEEDGGSSRSSDV

SEQ ID NO: 35 - DNA, 768 bp, Artificial sequence
  Synthetic: TRAP HMGB1 nucleotide sequence
ggatccatgggcggtagcagcagaagcagcgcagcacctgaaacgagagcagtccagccgaaacctgaagaaggccatgaaagacctgaacctgaagaagaagaagagaaaaaagaagaaggcggcggctttcctacagcagcagtcgcgggcggatcaagcagatcttccatgggtaaaggcgacccgaaaaaacctcggggcaaaatgtcaagctacgcatttttcgtccaaacatgcagagaagaacataagaaaaaacatcctgatgctagcgtaaacttttcagaatttagcaaaaaatgttctgaacgttggaaaacgatgtcttccaaagaaaagggtaaatttgaagatatggctaaagccgacaaattgcggtacgaaaaagaaatgaaaaactacgtaccgcctaaaggagaaacaaagaaaaaatttaaagatccgaacgcccctaaaagaccgccttctgcatttttcctgttttgctccgaatttcgcccgaaaattaaaggagaacatcctggtctgagcatcggcgacgttgcgaaaaaacttggagaaatgtggaataacacggcagcggatgacaaacagccgtatgagaaaaaagctgccaaattgaaagaaaaatacgaaaaagatatcgcagcgtaccgcgcaaaaggaaaagtggacgcgggtaaaaaagttgtggctaaagcggaaaaatcaaagaagaaaaaggaagaagaagaagacggcggctcatctcggtcctccgacgtc

SEQ ID NO: 36 - protein, 256 aa, Artificial sequence
  Synthetic: TRAP HMGB1 peptide
GSMGGSSRSSAAPETRAVQPKPEEGHERPEPEEEEEKKEEGGGFPTAAVAGGSSRSSMGKGDPKKPRGKMSSYAFFVQTCREEHKKKHPDASVNFSEFSKKCSERWKTMSSKEKGKFEDMAKADKLRYEKEMKNYVPPKGETKKKFKDPNAPKRPPSAFFLFCSEFRPKIKGEHPGLSIGDVAKKLGEMWNNTAADDKQPYEKKAAKLKEKYEKDIAAYRAKGKVDAGKKVVAKAEKSKKKKEEEEDGGSSRSSDV

SEQ ID NO: 37 - protein, 32 aa, Toxoplasma gondii
  misc_feature (1)..(32): Toxoplasma gondii RH
PRVISFGYGACEHNLGVSLFRREETKKDPRGR

SEQ ID NO: 38 - protein, 43 aa, Artificial sequence
  Synthetic: Consensus sequence
  misc_feature (11)..(11): Xaa can be any amino acid
  misc_feature (13)..(17): Xaa can be any amino acid
  misc_feature (24)..(24): Xaa can be any amino acid
  misc_feature (28)..(28): Xaa can be any amino acid
  misc_feature (31)..(32): Xaa can be any amino acid
  misc_feature (35)..(39): Xaa can be any amino acid
PSHDAPESZRXPXXXXXGYGACEXNLGXSLXXRZXXXXXPRGR

SEQ ID NO: 39 - protein, 841 aa, Toxoplasma gondii
  misc_feature (1)..(841): Toxoplasma gondii ROM5
MSSKGGSSRLGSKDLKKMTSRTERELRDSGRVRGEVERVEKRLRATAKVKEQPPTGDYKRRALASPGETAAPTFLVDSRGIPRKTSSTAPRKATLRPASSSPRLASSSRPTESTLPSSSSRALQGASSSSSSRPRRLHESASGRGGSGGSAGELRQEKKRLPELEAAEAAPASCVVELRDVTARKGRTSPATPPETAGSSVCGQGSHARTAEKLEEGTASHRDGSRRGSVDAETWATPGDGSSSHEFESSPQREERMQPQETGRRELSSEPRSGDLTKNGGDGGPRRHSCAWRKWREHMIQSFDITTHPFPPRGDGSPRRGKFLMIFLTSSVLFFVFLQELVLNVTTFNGRCMSPVLYPSHDAPESERTPRVISFGYGACEHNLGVSLFRREETKKDPRGRWTPGPLTERCASGRCASDDGWPSDLVQRGRAQRSPAAFDSPNPRVFSSLGALDTNKVRNYGEMFRVVWGMFLHGGWMHLLLNVSCQAQTLWILEPAWGFLRTLSLWIVGGVSGSLLSAVANPCTVTVGSSGAFYGLLGALVPFSIEYWDHIASPAWFLFCVSVLVMVAQFGNMVGVQGVDNNAHLGGLIGGLLFGFATIRSVHAFRWQGVAERMASSTLFWWMFPAEKRRSLREDNLQRVAREREERSSGRIPPPKFVWKFRGHEREWCVRFAAAVGLVTFWSVLWLYLLVPSYYESLSSPPGNFSFLGSTGCHCCRVQPFPGEEDKLPAFHPVRVNRGLFWCFVSEGVANLFCGRSSALNRGADVYGQTRQFEEALGDLPSARAGEAPLRIAKEEGESASVWQRLVKSAKKTYNAVLGNTTTPAAPSAAELAQQTRAGQ

SEQ ID NO: 40 - protein, 40 aa, Eimeria maxima
  misc_feature (1)..(40): Eimeria maxima TRAP-02A
AAPETRAVQPKPEEGHERPEPEEEEEKKEEGGGFPTAAVA